European Patent Application EP 4 455 288 A1, published October 30, 2024. Title: Enzyme, complex, recombinant vector, therapeutic agent for genetic disorder and polynucleotide. Applicant: Japan Advanced Institute of Science and Technology. Application WO. The sequence listing filed with the application follows.

SEQUENCE LISTING (13 sequences)

SEQ ID NO: 1 - protein, 171 aa, synthetic construct
PKNAATYVLLSNIYAEAGKWDMVSWVRTMMRERGIRKKKPAVATVEVNKEVHRFLVGEMREDIALKVESTNARLKQEGGHVPHTELVLKPLSQKEKEDMLCGHAEKLALAFGLLNTPSGTPLVVTKNLRMCNDCHSSTKIMSRVEQRDIVVRDGYRVHRFTNGCCSCKGRP

SEQ ID NO: 2 - protein, 171 aa, synthetic construct
PKNAATYVLLSNIYAEAGKWDMVSWVRTMMRERGIRKKKPAVATIEVNMEVHRFLVGERREDIALKLESTNARLKQEGGHVPHTKLVLKPLSEKEKEDALCGHAEKLALAFGLLNTPSGTPLVVTKNLRMCSDCHSSTEIMSRLEQRDIVVRDGYRVHRFANGCCSCKGRP

SEQ ID NO: 3 - protein, 37 aa, synthetic construct
PKNAATYVLLSNIYAEAGKWDMVSWVRTMMRERGIRK

SEQ ID NO: 4 - DNA, 202 bp, synthetic construct
  misc_feature 1..202: note = Nad4 mutant
  misc_feature 1..21: note = n is a, c, g, or t
  misc_feature 30: note = n is a, c, g, or t
  misc_feature 190: note = n is a, c, g, or t
  misc_feature 199: note = n is a, c, g, or t
  misc_feature 201: note = n is a, c, g, or t
  source 1..202: mol_type = other DNA
nnnnnnnnnnnnnnnnnnnnntcgggctcntgagcgcttgtttcggcgtgggtatggtggcaggccccgtggccgggggactgttgggcgccatctccttgcatgctcaaacatcaatttttatataggtatagacggtatctctttattttgtcgaccgatgcccttgagagccttcaacccagtcacnccttccggntnt

SEQ ID NO: 5 - DNA, 19 bp, synthetic construct
  misc_feature 1..19: note = Forward primer
  source 1..19: mol_type = other DNA
aatctaacaatgcgctcat

SEQ ID NO: 6 - DNA, 18 bp, synthetic construct
  misc_feature 1..18: note = Reverse primer
  source 1..18: mol_type = other DNA
accggaaggagctgactg

SEQ ID NO: 7 - RNA, 21 nt, synthetic construct
  source 1..21: mol_type = other RNA
cactgcacgccgttggtcagg

SEQ ID NO: 8 - protein, 312 aa, synthetic construct
MKVRNVVSWNAMISGLAQHGLGQDALEVFRRMTAHGVKPDRVTFVAVLSACSHAGLVDEGRSQYLAMTQVYGIEPDVSHCNCMVDLLGRAGRLMEAKLFIDNMAVDPDEATWGALLGSCRTYGNVELGELVAKERLKLDPKNAATYVLLSNIYAEAGKWDMVSWVRTMMRERGIRKEPGRSWIEVDNKIHDFLVADSSHPECKEINESKDKVIEKIKAEGYIPDTRLVLKNKNMKDKELDICSHSEKLAIVYGLMHTPPGNPIRVFKNLRVCTDCHGATKLISKVEGREIIVRDANRFHHFKDGVCSCGDYW

SEQ ID NO: 9 - protein, 280 aa, synthetic construct
TAHGVKPDRVTFVAVLSACSHAGLVDEGRSQYLAMTQVYGIEPDVSHCNCMVDLLGRAGRLMEAKLFIDNMAVDPDEATWGALLGSCRTYGNVELGELVAKERLKLDPKNAATYVLLSNIYAEAGKWDMVSWVRTMMRERGIRKEPGRSWIEVDNKIHDFLVADSSHPECKEINESKDKVIEKIKAEGYIPDTRLVLKNKNMKDKELDICSHSEKLAIVYGLMHTPPGNPIRVFKNLRVCTDCHGATKLISKVEGREIIVRDANRFHHFKDGVCSCGDYW

SEQ ID NO: 10 - protein, 246 aa, synthetic construct
MTQVYGIEPDVSHCNCMVDLLGRAGRLMEAKLFIDNMAVDPDEATWGALLGSCRTYGNVELGELVAKERLKLDPKNAATYVLLSNIYAEAGKWDMVSWVRTMMRERGIRKEPGRSWIEVDNKIHDFLVADSSHPECKEINESKDKVIEKIKAEGYIPDTRLVLKNKNMKDKELDICSHSEKLAIVYGLMHTPPGNPIRVFKNLRVCTDCHGATKLISKVEGREIIVRDANRFHHFKDGVCSCGDYW

SEQ ID NO: 11 - protein, 210 aa, synthetic construct
MAVDPDEATWGALLGSCRTYGNVELGELVAKERLKLDPKNAATYVLLSNIYAEAGKWDMVSWVRTMMRERGIRKEPGRSWIEVDNKIHDFLVADSSHPECKEINESKDKVIEKIKAEGYIPDTRLVLKNKNMKDKELDICSHSEKLAIVYGLMHTPPGNPIRVFKNLRVCTDCHGATKLISKVEGREIIVRDANRFHHFKDGVCSCGDYW

SEQ ID NO: 12 - protein, 173 aa, synthetic construct
PKNAATYVLLSNIYAEAGKWDMVSWVRTMMRERGIRKEPGRSWIEVDNKIHDFLVADSSHPECKEINESKDKVIEKIKAEGYIPDTRLVLKNKNMKDKELDICSHSEKLAIVYGLMHTPPGNPIRVFKNLRVCTDCHGATKLISKVEGREIIVRDANRFHHFKDGVCSCGDYW

SEQ ID NO: 13 - protein, 139 aa, synthetic construct
IRKEPGRSWIEVDNKIHDFLVADSSHPECKEINESKDKVIEKIKAEGYIPDTRLVLKNKNMKDKELDICSHSEKLAIVYGLMHTPPGNPIRVFKNLRVCTDCHGATKLISKVEGREIIVRDANRFHHFKDGVCSCGDYW